European Patent Application EP 4 737 577 A1, published May 6, 2026. Title: 一种CFB基因修饰的非人动物. Applicant: 百奥赛图（北京）医药科技股份有限公司. The sequence listing filed with the application follows.

SEQUENCE LISTING (59 sequences)

SEQ ID NO: 1 - protein, 763 aa, Mus musculus
MTMESPQLCLVLLVLGFSSGGVSATPVLEARPQVSCSLEGVEIKGGSFQLLQGGQALEYLCPSGFYPYPVQTRTCRSTGSWSDLQTRDQKIVQKAECRAIRCPRPQDFENGEFWPRSPFYNLSDQISFQCYDGYVLRGSANRTCQENGRWDGQTAICDDGAGYCPNPGIPIGTRKVGSQYRLEDIVTYHCSRGLVLRGSQKRKCQEGGSWSGTEPSCQDSFMYDSPQEVAEAFLSSLTETIEGADAEDGHSPGEQQKRKIVLDPSGSMNIYLVLDGSDSIGSSNFTGAKRCLTNLIEKVASYGVRPRYGLLTYATVPKVLVRVSDERSSDADWVTEKLNQISYEDHKLKSGTNTKRALQAVYSMMSWAGDAPPEGWNRTRHVIIIMTDGLHNMGGNPVTVIQDIRALLDIGRDPKNPREDYLDVYVFGVGPLVDSVNINALASKKDNEHHVFKVKDMEDLENVFYQMIDETKSLSLCGMVWEHKKGNDYHKQPWQAKISVTRPLKGHETCMGAVVSEYFVLTAAHCFMVDDQKHSIKVSVGGQRRDLEIEEVLFHPKYNINGKKAEGIPEFYDYDVALVKLKNKLKYGQTLRPICLPCTEGTTRALRLPQTATCKQHKEQLLPVKDVKALFVSEQGKSLTRKEVYIKNGDKKASCERDATKAQGYEKVKDASEVVTPRFLCTGGVDPYADPNTCKGDSGGPLIVHKRSRFIQVGVISWGVVDVCRDQRRQQLVPSYARDFHINLFQVLPWLKDKLKDEDLGFL

SEQ ID NO: 2 - protein, 764 aa, Homo sapiens
MGSNLSPQLCLMPFILGLLSGGVTTTPWSLARPQGSCSLEGVEIKGGSFRLLQEGQALEYVCPSGFYPYPVQTRTCRSTGSWSTLKTQDQKTVRKAECRAIHCPRPHDFENGEYWPRSPYYNVSDEISFHCYDGYTLRGSANRTCQVNGRWSGQTAICDNGAGYCSNPGIPIGTRKVGSQYRLEDSVTYHCSRGLTLRGSQRRTCQEGGSWSGTEPSCQDSFMYDTPQEVAEAFLSSLTETIEGVDAEDGHGPGEQQKRKIVLDPSGSMNIYLVLDGSDSIGASNFTGAKKCLVNLIEKVASYGVKPRYGLVTYATYPKIWVKVSEADSSNADWVTKQLNEINYEDHKLKSGTNTKKALQAVYSMMSWPDDVPPEGWNRTRHVIILMTDGLHNMGGDPITVIDEIRDLLYIGKDRKNPREDYLDVYVFGVGPLVNQVNINALASKKDNEQHVFKVKDMENLEDVFYQMIDESQSLSLCGMVWEHRKGTDYHKQPWQAKISVIRPSKGHESCMGAVVSEYFVLTAAHCFTVDDKEHSIKVSVGGEKRDLEIEVVLFHPNYNINGKKEAGIPEFYDYDVALIKLKNKLKYGQTIRPICLPCTEGTTRALRLPPTTTCQQQKEELLPAQDIKALFVSEEEKKLTRKEVYIKNGDKKGSCERDAQYAPGYDKVKDISEVVTPRFLCTGGVSPYADPNTCRGDSGGPLIVHKRSRFIQVGVISWGVVDVCKNQKRQKQVPAHARDFHINLFQVLPWLKEKLQDEDLGFL

SEQ ID NO: 3 - DNA, 3608 bp, synthetic construct
  source 1..3608: mol_type = other DNA
acattttttttatgtgtgtgtgtgtgtgtgtgagagattgtgagtgcctttggaagctggaggaggacatcacctcccctggaactggagttacagtcgatggtgctggagcctgaactccagtcctctggaagcgcggcaagcactgaccactgagcattcagccctcttttgttttcttttggggatgggcccaggttggcctccaactcaagaggtagcctaggctgatgttcctaactccacctcctgaggcaaaagaccctgggggggcaaatgcctttaacttcagcacttgggaggcggaggcatgaggatctctgtgagttcgaggccagcctgatctacaaagtaagttccaagacagccagagctacacagagacactgtctccaaaagaaaaaaaaaaagaccctaattctaattcaggtcacatccacaatagaatagaacttgaacacatccttctggggacacacaattctacccactgcaggcaaacacaaaagagaaacaaggcagcccgttagcattctagtggtgacatgatgtgaagccaagtgggggtggcatgggagggtctggggcattgcagcctgggggagagcaccccagccagaggtgcagctggagcagaggcctgaggaaggaatgtacatgctggtttgaggagcttctaagaggctggggcatggggggctgagtggcagtaggagaggaagcgagccggagtgaaggagatggagcccatctaactcaggcctttgtcagctggtgagttcaagtacccacttcctgtctcaggtggcctctcagtcacaggctctggtgatttccctccttcccaccagacatctatgctattggggtgggcaagctggatgtggactggaaagaactgaatgagctgggttccaagaaggatggcgagaggcatgccttcatcttgcaggatgcaaaggccttgcaacagatctttgagcacatgttgggtgagtaagctttgtcccccgctgcagaagagagcatagtggggactcagatggggtctcacagtggcagcctggaccagtggcccttacccacttccctccccatcttcctttgcccatagatgtctctaagctcacagataccatctgtggggtggggaacatgtccgccaatgcctctgaccaggagaggacaccttggcaagtcacctttaaggtatcaggaaggagggacagggcttaggcatcagaggtaaaaacagccaggcacagcaaacccggattgttgtctcttccctgcagcccaagagcaaggaaacttgccagggatcactcatctctgatcagtgggtgctgacagcagctcactgcttccatgacattcagatggaggaccaccacctgtggagggtcaatgtaggtaagtcaggggctgcagtagatccctcactgcaaggccagagtcaccactgtctctcctcagcctttggtccagtctaattcacctttgtttccaggtgatcccacctctcagcatggcaaagaatttcttgtggaggacgtgataattgccccagggtttaatgtccatgcaaagcggaagcagggcatctcagagttctatgctgatgacattgccttgctgaagctatctcggaaagtgaaaatgtccacccatgccaggtgcctgaacccagatgggagagtaccctatagaggatggtgctctggaaagcaccagaggggatactgaggatgggcctgtttgacacttggctttctccccagacccatctgccttccttgcactgtgggagccaacatggctctgcggagatccccaggtagtacctgtaaagatcatggtgagtgctggaggcttgaggttcttggtgggttgcagccagagcttgcagggatcaggttcttgcagagtgccagcagggaccgggctgcagtcctcaagctgagtaaagaaatctgtaccaacacccacttctccccaatggcagagacagaacttctgtcacagcagaaagttcctgcacattttgtagctttgaatgggaacagactcaacatcaacctcaggacaggacctgaggtgagagcttagtaagggatgctgggataccctggaggcagctcccagaatgtccagccctgcctggagtctcgattcttggaccttacaggtctgcctaatgtctcctggaatgtcctcattcttctctcctatgccccacaccgcagtggacaaggtgtatccaggctgtctcccaaaacaaaaacatcttccccagcttgacaaacgttagcgaggtggtgacagaccagttcctatgcagtgggatggaggaggaagatgacaatccttgcaaaggttagtctgatcctggacttccagggagaaggctacggtgtccctgtaaccggttagcaagcactccaaatgctagtgtactgttctggacaatactgtcttttctttccctgaaggagaatctgggggagccgttttccttggacggagatacaggttcttccaggtgagaagcaggacccggaggggcctccctgccagggcacaagttcttcttgctgggggcaagtgggaggcctttgagaggaaccagagaggtcgaggcttagagtggggccaccactatctccaccctgttgtctcttccctccaggtgggcctggtgagttggggtctttttgacccttgtcatggttcctccaacaaaaacttgcgcaagaaacctccacgtggtgttctgccaagggacttccacattagtcttttccgcctgcagccctggctgaggcagcacctggatggtgtcctggactttctgccactttaacatggtcactgactcctttattagtctgaacttcctgtctaatacctctgagcgttctcactcctggatacataaatcttgggccccgggagcccagagacagtggcaaaagctagggaatccccaggattgtgccgggacctctgtgccacctgtgaagcaagtctctctctagtgtggatgacccgtgctccttttgctttcacacggaatttcccagttatgtaattaataaaaatcaatgatttccacatcctgtctgtcttatgtcttggggggtggggaggccaggaagattccaggaaggtcagagtccttgctgcacaaacagtggatggactttgctccatcacacagtccatggaaagactgatcttttaaattgggggtagtggaggtggtggtctgtgcttgttaggaggggtctgggggctaagagggagctttgaaagggaagttctggcccttggtcagtcaagggtggggctcacatagtttctgtttcctcagttggcagttcagctggggccctccttcatgaatgttccgggaagcagtggctgcgtgcgcagggtaggctggccaggctgcagatgccagagcagattgcataaaaggttaggggacagtgggaaaggggtgtagccagatccagcatttgggtttcagtttggacaggaggtcaaataggcacccagagtgacctggagagggctttgggccactggactctctggtgctttcc

SEQ ID NO: 4 - DNA, 3869 bp, synthetic construct
  source 1..3869: mol_type = other DNA
ttaacttgggcctagcaagccaggactgctggaggtatgctaggcacagacagtagagcctagcttcctaatgctcttgattctctaaaccagtctcaggtcacttttcaatctccaaaatccccacctctgatggttccagatacacagaacactaatctatgtttccatgcctggtcttctacttgaggtccagacccacaataccaagttcaggtaacactccagctcagaggcgacaactaggcttctgctttcctgtctgtgacagaggaccctgttctgtttttccaaatggcttttcttttctttctttttttttttttggttttctgagacagggtttctctgtgtagtcttggctgtcctggaactcactctgtagaccaagctggccttgaactcagaaatccaccttcctctgcctcccaagtgctgggattaaaggtgtgtgccaccactgccctgcccaaatggcttttcaagacaagatttctctgtgtagccctggctgttctgaactctgctctgtagaccaggctggccttgaactcacctggctccacctcccacgtgttgtggctgaaggtgtgtgccaccactgagagggcacatttcagtgctgctctccttccctcacctgacagatgccctggcaattcttcatccactacctacgtgaagatcctgaccttgggcactttagggaactcaaggaagtgctatgctgcagagaggggaagggaggagcctcatccttaccaagggagccccagacagatttgccagtagcagcgtccagcatgggctgttttcgggctatgttgactttaagctgcacagattccacctgggtcccattgagctgtgggacaagaggggaggggacagaggacgggcattacatggagccaggtgctgctgccctgggagaccaaccaggaatgtgaggatgaaggttttctcagtcaggagaaaagtttcctctagaagcagatattgaaaagaagaagcaggaggatgacaggagggatgggaggaacggtctgagaagtcccaacctcagcaacagcctgatctgcagactccatcttctcgtaggtgacgaaggcacagctgggtgagagagaaagcagagtcaggaaactccatggagaccaggcagctccctccccgggatgttgctcatgcttactttctgggtgggtccatggagaggtcgatgatatttccaaagggagagaaggccccgcggaggagggtgggcgtcatgtcctctccatacacatacagtgtgttcccctttcgaggggccctccgttcggggaatgagtctgaccctgtgggttaggaaccacagtcattactgggtccacctcaccttctacttagcaggacccacctaaaccctggctaagatcactcactgcggaaagggccctctcggtctcgttcccgatctcggtcccggtctctgtctcgatcccggtctctgtctttgtctttatcccggtctctgtctcgatctcgatctcggtctctgtctctctctttgtcccgatccctatctcggctccggtcatgacttcggtccctgctgcggcttcggggaggggaggctgaggagcgggcgctaccatgctcttcatagctccagtcaaagcctcgaggtgggccatcaccagccccgggggcctctgcttcttctccatcttgtcccagttcccgaagccgatcactagaagacacaaagctggggagaggcagacagtaaggaccaaagggggttcgaccttcttccaaaccttgtggagtcaacactgcctctgcagctggctcctcccactctagccctgaactttccagtcactctggcctctgaccccacaccaaacggtgctctctctgacctttcatacagagatttcctctggggacgtctggatggctaaggggaaagaaaagacagagaacaattcaaatgattcccaggtgccggagttggtccacagtgtgtgggtctcttcttgtccccaaccctggccccacagaaaccattacctcctgtaggtcctcatcagcagacatgctcctctggaacggctggaaagtggggacaggccccttctctgggtcctggaaaagggcagatacccatgttagcgtggatcaggagagctcttccctctctcttctctgcttctcttttgctcctgtcactcttatgatgatgtgctggaccggttgactggtttttcaagatagtgcttctctgtgtggccctggctatcctgaacttgcgcagtagaaccaggctgtcctttatgttagagctctcggcctgtctgctccaagtgctgggattaaaggtgtgtgccactacatcagctgatgtgagtaactggtttcattactcaaacctcccttcaatccaagaagcacaaatatggaaaagagatgtgggcatcacccaggctttttttttttgttttgtttttttttgttttgtttttcgagacagggtttctctgtatagccctggctgtcctagaactcactctgtagaccgggctggcctcaaactcagaaatctgcctgcctctgccccacaagtgctgggattaaaggcatgtgccaccacactgggctcaggtttctttgtgatagacagaaacctagcgctccagtgggctgcagtggcaaaaactacttctgaggctgaggccagagcatcacttgactccatgagtacagtcagaccctgtctcaaggaacaagaaagaaacaccctaaactcagaacagcacaggttgctcatatgtgagcatgcatgacttcccccacccacccccttccagctgatgccaggacgttccagacaatcttcctgtgtgctcacctttaacttcccttccagggtccgagaacgtttgaagcctgagttcttagtttcagccttgatggcactgatggctcctgacttcaccagttgtttggcctgttctgttgctgtggcagtgtccaccacaggctgctctgacagtgctggggagagagggagggggaaggagagaggcattcattatgctggctgtggagggaagccctctgctgctgccccctggactctctgtctctgtcacttacagcgtttgacaccgccctggctcgctgggccgctgctgctctgcttcttcagagccagcaatgcctttttctggaaaggagagaggtctgtcaaccagggtctggttccagggccagtgtgtgtggcatcctggtcctggagtggctcatcctgcttccacatcctcacgaagcccacagtacttaacctaaccaaactatggtgtccaaggccttccagtctcacattttggaaactgaaaaccaaaaacacctaagccctaccatataagctgcaaataagacctgaatccttggggattttatccacccatctcccatcttctgcacatttaatgaggccatgcagaatcaaaacacatagttcccacccttaaggaattcagaacccaggaaacaatggctagactgacagccaagaataatcaagggcactaatcactcagggctgagtataagcaacactttctgatgcataagcagctagtaaactgagacctcacagaattacccaacacagacagaaaagatactttagacaaagaaattggggttgcaaaaatgcagaggaggttttggaaggcaggttttaagagaaaataattctctcttttgacaggtatggtgagctgatatttcaattctatacatgatgtgaaacctcggaagtgttttcaatggatcaggtgtgccttcaaaacagcaaagccagaccctgtcaa

SEQ ID NO: 5 - DNA, 1451 bp, synthetic construct
  source 1..1451: mol_type = other DNA
tgcctggagtctcgattcttggaccttacaggtctgcctaatgtctcctggaatgtcctcattcttctctcctatgccccacaccgcagtggacaaggtgtatccaggctgtctcccaaaacaaaaacatcttccccagcttgacaaacgttagcgaggtggtgacagaccagttcctatgcagtgggatggaggaggaagatgacaatccttgcaaaggttagtctgatcctggacttccagggagaaggctacggtgtccctgtaaccggttagcaagcactccaaatgctagtgtactgttctggacaatactgtcttttctttccctgaaggagaatctgggggagccgttttccttggacggagatacaggttcttccaggtgagaagcaggacccggaggggcctccctgccagggcacaagttcttcttgctgggggcaagtgggaggcctttgagaggaaccagagaggtcgaggcttagagtggggccaccactatctccaccctgttgtctcttccctccaggtgggcctggtgagttggggtctttttgacccttgtcatggttcctccaacaaaaacttgcgcaagaaacctccacgtggtgttctgccaagggacttccacattagtcttttccgcctgcagccctggctgaggcagcacctggatggtgtcctggactttctgccactttaacatggtcactgactcctttattagtctgaacttcctgtctaatacctctgagcgttctcactcctggatacataaatcttgggccccgggagcccagagacagtggcaaaagctagggaatccccaggattgtgccgggacctctgtgccacctgtgaagcaagtctctctctagtgtggatgacccgtgctccttttgctttcacacggaatttcccagttatgtaattaataaaaatcaatgatttccacatcctgtctgtcttatgtcttggggggtggggaggccaggaagattccaggaaggtcagagtccttgctgcacaaacagtggatggactttgctccatcacacagtccatggaaagactgatcttttaaattgggggtagtggaggtggtggtctgtgcttgttaggaggggtctgggggctaagagggagctttgaaagggaagttctggcccttggtcagtcaagggtggggctcacatagtttctgtttcctcagttggcagttcagctggggccctccttcatgaatgttccgggaagcagtggctgcgtgcgcagggtaggctggccaggctgcagatgccagagcagattgcataaaaggttaggggacagtgggaaaggggtgtagccagatccagcatttgggtttcagtttggacaggaggtcaaataggcacccagagtgacctggagagggctttgggccactggactctctggtgctttcc

SEQ ID NO: 6 - DNA, 1577 bp, synthetic construct
  source 1..1577: mol_type = other DNA
agagcttcctgcagggagagtgtgaggacagattaaagcagttacaataacaagtgtgttccacatctttttggggtaagggcgtgcactggttaacatcaacactgacagccgcttttgaaggcttaactccaatcccaagtgctgaaagactagaggctgacggaggtgaaaagcttctaccccaggattttactgagaccagcttgggggcatatgaggcacaaggaatccagcttcatgtcctagaagccatccacaaggtttcctatagatcgtcactgtacacaatctgggtcctcttgtctcgatggcaacccttagggctgttctggacagctaaggagggaggaaagtgacagttaagtgaagcaccagtggcgttagacctggggtccagagccctggccctggtccaccagggcttactctgccctctggtggccataacctcactgtggcttagaaaatccagaatgttaacacagttagagatgtgactatgataacatcacaaatacatggaaattaaaagatcagaatgtttctgtaccttgctggtacactggtcaattctggttccttcctagtgtgtgcaaggactttgcttactccttcctcagaaaagtttgttttgggtagaatgggctgtccacactgagagaccccatgaggacctctccgaactcaagtgttcagcttttctttcctcatactgctcatccctcccaaggattccctgtggggctaagagacaggcctcctctttggtcttatactcttttcagagcctctcagcccacagcccagagcttctggggttgttcttagcttggactcttcttcatggctcctttgctgcagacttaacttgggcctagcaagccaggactgctggaggtatgctaggcacagacagtagagcctagcttcctaatgctcttgattctctaaaccagtctcaggtcacttttcaatctccaaaatccccacctctgatggttccagatacacagaacactaatctatgtttccatgcctggtcttctacttgaggtccagacccacaataccaagttcaggtaacactccagctcagaggcgacaactaggcttctgctttcctgtctgtgacagaggaccctgttctgtttttccaaatggcttttcttttctttctttttttttttttggttttctgagacagggtttctctgtgtagtcttggctgtcctggaactcactctgtagaccaagctggccttgaactcagaaatccaccttcctctgcctcccaagtgctgggattaaaggtgtgtgccaccactgccctgcccaaatggcttttcaagacaagatttctctgtgtagccctggctgttctgaactctgctctgtagaccaggctggccttgaactcacctggctccacctcccacgtgttgtggctgaaggtgtgtgccaccactgagagggcacatttcagtgctgctctccttccctcacctgacagatgccctggcaattcttcatccactacctacgtgaagatcctgaccttgggcactttagggaac

SEQ ID NO: 7 - DNA, 5809 bp, synthetic construct
  source 1..5809: mol_type = other DNA
atggggagcaatctcagcccccaactctgcctgatgccctttatcttgggcctcttgtctggaggtaagcgagggtaaccttcccttcctgctgtctccagcatccctccttggccttttggggccaggcttcatcagcctttctcttcaggtgtgaccaccactccatggtctttggcccggccccagggatcctgctctctggagggggtagagatcaaaggcggctccttccgacttctccaagagggccaggcactggagtacgtgtgtccttctggcttctacccgtaccctgtgcagacacgtacctgcagatctacggggtcctggagcaccctgaagactcaagaccaaaagactgtcaggaaggcagagtgcagaggtttgagggcaatgagtgtgggcagtggcctaaggcagaaacagggcaggcggcagcaaggtcaggactaggatgagactaggcagggtgacaaggtgggctgaccgggagtaggagcagttttagggtggcaggcggaaagggggcaagaaaaagcggagttaacccttactaagcatttaccctgggcttccaggcagccctggaagtcaagagaacactcagaaatggggagggagaagcagtggaaatccatatgggttgaggagtaggtaagatgctgcttctgcgggactgggaatgcgctgtttctcagtgacatggtctccgagaccaggagggatacacctaaggcagcctttccctcttgatgacttctacttgtccccccttctcaaagcaatccactgtccaagaccacacgacttcgagaacggggaatactggccccggtctccctactacaatgtgagtgatgagatctctttccactgctatgacggttacactctccggggctctgccaatcgcacctgccaagtgaatggccgatggagtgggcagacagcgatctgtgacaacggaggtgagaagcatcccctccccctacattgctgtctccctgacggcgcccagcccgaggagtgggcactcggctccggacactgtaactcttgctctctaccttgctcacggggcctcaggcttcagtgcttacctcgatgtctcatacctctgcagcggggtactgctccaacccgggcatccccattggcacaaggaaggtgggcagccagtaccgccttgaagacagcgtcacctaccactgcagccgggggcttaccctgcgtggctcccagcggcgaacgtgtcaggaaggtggctcttggagcgggacggagccttcctgccaaggtgacctttgacctgtacccccaggtcagatcctggtcttccatcctactgtcttctctccccacctcaaccctgctctttcctcactttgtttaaacctccctgtacaactatctcacttctgagccttttataccctggaaacccatgatcccccgtctctttggtcactgtatccctgacactcccagacatttgacctcatttctgactctcccagactccttcatgtacgacacccctcaagaggtggccgaagctttcctgtcttccctgacagagaccatagaaggagtcgatgctgaggatgggcacggcccaggtttgaagacagagaagggaggcagggcagggaactgggggaaaatggagaagggacagaactgttaatgctggagcctgagccactctcctggcacccaggggaacaacagaagcggaagatcgtcctggacccttcaggctccatgaacatctacctggtgctagatggatcagacagcattggggccagcaacttcacaggagccaaaaagtgtctagtcaacttaattgagaaggtggaatcctcctatccctgaactcgggggaatggaatctcgctgatcttccaggactagctccctgatcattccagcccctctgaacaacagggccccaggaaaatctccaggtcctattctgtcctccttcccttttacttgaagcagtttcttgactggtaattcctccatgaacctcagcccttgagcctcttactgagagcctccctgtcccagcaaagtcgctgaaatctcccaatcacagtattctattttcaatgccatggcgccttgttctcctcacccacaggtggcaagttatggtgtgaagccaagatatggtctagtgacatatgccacataccccaaaatttgggtcaaagtgtctgaagcagacagcagtaatgcagactgggtcacgaagcagctcaatgaaatcaattatgaaggtcagaggttagggaatggtgggaggttcactttggggtcaggaggttcagggtggagggggtcatgagactaccttgagggcgacagggaggaccactttgtagtcaaaagttgaacagcaggatcgttgggcaatggaggttagtgggaacctgttgggggctggaagggccactttgtggtcaaagggaagtccgtgtaatgatgattaacttaaaaagttgaaagatgtgggatttcagttgcagattggtctctggggttaaaagatggcttggaagaccaggtgaggtgatggtctcttccctctccacagaccacaagttgaagtcagggactaacaccaagaaggccctccaggcagtgtacagcatgatgagctggccagatgacgtccctcctgaaggctggaaccgcacccgccatgtcatcatcctcatgactgatggtcagaagggacctctctcctgtcccagcctccccaccttctcagaccagcatgtggcccttaagtccacttgtaacactatacccatggttggggccctgaatgtgactcatagctggctgttcatctctcctgtgacccttcataaggaattcttcctaagccctgtgatcaactatctctaacccttcctcaacttgctcaccctgccatgtgtatccctgcctttagccagtttatcttccttatctcctaccctcatggtcctgtctcttctgcaggattgcacaacatgggcggggacccaattactgtcattgatgagatccgggacttgctatacattggcaaggatcgcaaaaacccaagggaggattatctgggtgagtaacctgcctaggacccagcaccccacttcctcagggcttggaccctcatccttcctttttatccctcagatgtctatgtgtttggggtcgggcctttggtgaaccaagtgaacatcaatgctttggcttccaagaaagacaatgagcaacatgtgttcaaagtcaaggatatggaaaacctggaagatgttttctaccaaatgatcggtagggagatacaagggaataaagaacacaactctcctcaggttcccctgaagtaattcattcttcctctacacctgaagctctagttgcctggaaagccttcttcattcctccttctctacctcagtgtcactattcttgtttcctggcactgttcacttaaccttagaatcacagagctctgagcacttcagagatctttctatagtcctacatttgacacgtggaaacagaagccaaaggaggtcaagggacagcaagttagcaacaagggtgggcttgaaaacagccaggcctctgacagcttgatcccaagttctttcccttttcagtccaccatagcagttttctcctaacacgaggaaacaaatacccgtggtctttccctttctccttttgggcctttgctccccatagactcctacccaaaaggctgctgccatttgggaatgaagtgttccgagttttcagcacattctccttctctgccagatgaaagccagtctctgagtctctgtggcatggtttgggaacacaggaagggtaccgattaccacaagcaaccatggcaggccaagatctcagtcattgtaagcacagaatcccagtagtggggacttgggggaggtgaggtcaaggtgaaatgggagtaggggaaggaaaaaatggccataagagatggtggtttgtgaaagttgagctttccctctctactgttgtgtccccagcgcccttcaaagggacacgagagctgtatgggggctgtggtgtctgagtactttgtgctgacagcagcacattgtttcactgtggatgacaaggaacactcaatcaaggtcagcgtaggtaaggatgcaactgaaggtcctgggctgcacctatgctctccaggcaacacctcccactttctacagatcctacactccacccatcctcaatgcagccccattccttgcaccccagaccagtcagggatgggggaagacgtgaagttaggaatgacacggggccagaggcaggaagctgcccacaaagaggtggtacctactctcctacttcaggaggggagaagcgggacctggagatagaagtagtcctatttcaccccaactacaacattaatgggaaaaaagaagcaggaattcctgaattttatgactatgacgttgccctgatcaagctcaagaataagctgaaatatggccagactatcaggtgagagcgtccagatccctgaggaaaggctgggaaaggctggaggactggggtgaggagcaggcctggtttgctgttctccttgtcctttataggcccatttgtctcccctgcaccgagggaacaactcgagctttgaggcttcctccaactaccacttgccagcaacaaagtaagacatacttggcaagaggataaggatgagatcccaagagacaagtggggcatgagagggaggtgcaataggaagagatgatgcctggcccagaacctagctctagaagggcttaggggacatctactgagtgacaaaggcaatggggagatgacagtggtgggagcagctgaagtgacgcagtctattcgtccagaggaagagctgctccctgcacaggatatcaaagctctgtttgtgtctgaggaggagaaaaagctgactcggaaggaggtctacatcaagaatggggataaggtgagaaacgggcatcctaaggaggcactctaggccccaatccttcctaagccacttctgttcattacttctccatgcttcccacctcccctacagaaaggcagctgtgagagagatgctcaatatgccccaggctatgacaaagtcaaggacatctcagaggtggtcacccctcggttcctttgtactggaggagtgagtccctatgctgaccccaatacttgcagaggtgagagaatgctctttggttgtgctacaagtgcccaaggcccaacagtccttttctctacagcttctcctctccttgcaggtgattctggcggccccttgatagttcacaagagaagtcgtttcattcaagtgagtcctccctttcctatctggggagatgccaagtggtcagcatgggccccaaagcaggaaagctcaatgcatgtggctagtaattcgaggtaggcagagcctgcctcaccttaggaccgcatgtcttgcctgcgtgtgtcaagaacgaggctgagctgggtccctagtctgattcctttaggtcagctaagacacaagcaggaacagccatgcttccaggattaggaattctactgaatgatccatggcaccccactgcctctgcaggttggtgtaatcagctggggagtagtggatgtctgcaaaaaccagaagcggcaaaagcaggtacctgctcacgcccgagactttcacatcaacctctttcaagtgctgccctggctgaaggagaaactccaagatgaggatttgggttttctataa

SEQ ID NO: 8 - RNA, 2770 nt, synthetic construct
  source 1..2770: mol_type = other RNA
gctccatcacacagtccatggaaagactgatcttttaaattgggggtagtggaggtggtggtctgtgcttgttaggaggggtctgggggctaagagggagctttgaaagggaagttctggcccttggtcagtcaagggtggggctcacatagtttctgtttcctcagttggcagttcagctggggccctccttcatgaatgttccgggaagcagtggctgcgtgcgcagggtaggctggccaggctgcagatgccagagcagattgcataaaaggttaggggacagtgggaaaggggtgtagccagatccagcatttgggtttcagtttggacaggaggtcaaataggcacccagagtgacctggagagggctttgggccactggactctctggtgctttccatggggagcaatctcagcccccaactctgcctgatgccctttatcttgggcctcttgtctggaggtgtgaccaccactccatggtctttggcccggccccagggatcctgctctctggagggggtagagatcaaaggcggctccttccgacttctccaagagggccaggcactggagtacgtgtgtccttctggcttctacccgtaccctgtgcagacacgtacctgcagatctacggggtcctggagcaccctgaagactcaagaccaaaagactgtcaggaaggcagagtgcagagcaatccactgtccaagaccacacgacttcgagaacggggaatactggccccggtctccctactacaatgtgagtgatgagatctctttccactgctatgacggttacactctccggggctctgccaatcgcacctgccaagtgaatggccgatggagtgggcagacagcgatctgtgacaacggagcggggtactgctccaacccgggcatccccattggcacaaggaaggtgggcagccagtaccgccttgaagacagcgtcacctaccactgcagccgggggcttaccctgcgtggctcccagcggcgaacgtgtcaggaaggtggctcttggagcgggacggagccttcctgccaagactccttcatgtacgacacccctcaagaggtggccgaagctttcctgtcttccctgacagagaccatagaaggagtcgatgctgaggatgggcacggcccaggggaacaacagaagcggaagatcgtcctggacccttcaggctccatgaacatctacctggtgctagatggatcagacagcattggggccagcaacttcacaggagccaaaaagtgtctagtcaacttaattgagaaggtggcaagttatggtgtgaagccaagatatggtctagtgacatatgccacataccccaaaatttgggtcaaagtgtctgaagcagacagcagtaatgcagactgggtcacgaagcagctcaatgaaatcaattatgaagaccacaagttgaagtcagggactaacaccaagaaggccctccaggcagtgtacagcatgatgagctggccagatgacgtccctcctgaaggctggaaccgcacccgccatgtcatcatcctcatgactgatggattgcacaacatgggcggggacccaattactgtcattgatgagatccgggacttgctatacattggcaaggatcgcaaaaacccaagggaggattatctggatgtctatgtgtttggggtcgggcctttggtgaaccaagtgaacatcaatgctttggcttccaagaaagacaatgagcaacatgtgttcaaagtcaaggatatggaaaacctggaagatgttttctaccaaatgatcgatgaaagccagtctctgagtctctgtggcatggtttgggaacacaggaagggtaccgattaccacaagcaaccatggcaggccaagatctcagtcattcgcccttcaaagggacacgagagctgtatgggggctgtggtgtctgagtactttgtgctgacagcagcacattgtttcactgtggatgacaaggaacactcaatcaaggtcagcgtaggaggggagaagcgggacctggagatagaagtagtcctatttcaccccaactacaacattaatgggaaaaaagaagcaggaattcctgaattttatgactatgacgttgccctgatcaagctcaagaataagctgaaatatggccagactatcaggcccatttgtctcccctgcaccgagggaacaactcgagctttgaggcttcctccaactaccacttgccagcaacaaaaggaagagctgctccctgcacaggatatcaaagctctgtttgtgtctgaggaggagaaaaagctgactcggaaggaggtctacatcaagaatggggataagaaaggcagctgtgagagagatgctcaatatgccccaggctatgacaaagtcaaggacatctcagaggtggtcacccctcggttcctttgtactggaggagtgagtccctatgctgaccccaatacttgcagaggtgattctggcggccccttgatagttcacaagagaagtcgtttcattcaagttggtgtaatcagctggggagtagtggatgtctgcaaaaaccagaagcggcaaaagcaggtacctgctcacgcccgagactttcacatcaacctctttcaagtgctgccctggctgaaggagaaactccaagatgaggatttgggttttctataaagagcttcctgcagggagagtgtgaggacagattaaagcagttacaataacaaaaaaaaaaaaaaaaaaaaaa

SEQ ID NO: 9 - DNA, 86 bp, synthetic construct
  source 1..86: mol_type = other DNA
agggctttgggccactggactctctggtgctttccatggggagcaatctcagcccccaactctgcctgatgccctttatcttgggc

SEQ ID NO: 10 - DNA, 99 bp, synthetic construct
  source 1..99: mol_type = other DNA
tgctgccctggctgaaggagaaactccaagatgaggatttgggttttctataaagagcttcctgcagggagagtgtgaggacagattaaagcagttaca

SEQ ID NO: 11 - DNA, 90 bp, synthetic construct
  source 1..90: mol_type = other DNA
ggggttgttcttagcttggactcttcttcatggctcctttgctgcagacgtcgacggtatcgataagcttgatatcgaattccgaagttc

SEQ ID NO: 12 - DNA, 75 bp, synthetic construct
  source 1..75: mol_type = other DNA
tataggaacttcatcagtcaggtacataatggtggatccttaacttgggcctagcaagccaggactgctggaggt

SEQ ID NO: 13 - DNA, 23 bp, synthetic construct
  source 1..23: mol_type = other DNA
agcctaagaccaagaggacgagg

SEQ ID NO: 14 - DNA, 23 bp, synthetic construct
  source 1..23: mol_type = other DNA
gtggaagtcccgggcataagagg

SEQ ID NO: 15 - RNA, 20 nt, synthetic construct
  source 1..20: mol_type = other RNA
agcctaagaccaagaggacg

SEQ ID NO: 16 - RNA, 24 nt, synthetic construct
  source 1..24: mol_type = other RNA
taggagcctaagaccaagaggacg

SEQ ID NO: 17 - RNA, 20 nt, synthetic construct
  source 1..20: mol_type = other RNA
cgtcctcttggtcttaggct

SEQ ID NO: 18 - RNA, 24 nt, synthetic construct
  source 1..24: mol_type = other RNA
aaaccgtcctcttggtcttaggct

SEQ ID NO: 19 - RNA, 20 nt, synthetic construct
  source 1..20: mol_type = other RNA
gtggaagtcccgggcataag

SEQ ID NO: 20 - RNA, 24 nt, synthetic construct
  source 1..24: mol_type = other RNA
tagggtggaagtcccgggcataag

SEQ ID NO: 21 - RNA, 20 nt, synthetic construct
  source 1..20: mol_type = other RNA
cttatgcccgggacttccac

SEQ ID NO: 22 - RNA, 24 nt, synthetic construct
  source 1..24: mol_type = other RNA
aaaccttatgcccgggacttccac

SEQ ID NO: 23 - DNA, 132 bp, synthetic construct
  source 1..132: mol_type = other DNA
gaattctaatacgactcactatagggggtcttcgagaagacctgttttagagctagaaatagcaagttaaaataaggctagtccgttatcaacttgaaaaagtggcaccgagtcggtgcttttaaaggatcc

SEQ ID NO: 24 - DNA, 23 bp, synthetic construct
  source 1..23: mol_type = other DNA
ctgcagatgccagagcagattgc

SEQ ID NO: 25 - DNA, 25 bp, synthetic construct
  source 1..25: mol_type = other DNA
caagcactggagttgcgctcacacc

SEQ ID NO: 26 - DNA, 25 bp, synthetic construct
  source 1..25: mol_type = other DNA
ggtcttgagtcttcagggtgctcca

SEQ ID NO: 27 - DNA, 24 bp, synthetic construct
  source 1..24: mol_type = other DNA
gctcactgcttccatgacattcag

SEQ ID NO: 28 - DNA, 25 bp, synthetic construct
  source 1..25: mol_type = other DNA
gggttcaggcacctggcatgggtgg

SEQ ID NO: 29 - DNA, 24 bp, synthetic construct
  source 1..24: mol_type = other DNA
ctggggagatgccaagtggtcagc

SEQ ID NO: 30 - DNA, 23 bp, synthetic construct
  source 1..23: mol_type = other DNA
agctgattacaccaacctgcaga

SEQ ID NO: 31 - DNA, 20 bp, synthetic construct
  source 1..20: mol_type = other DNA
ctctggtggactccgtgaac

SEQ ID NO: 32 - DNA, 20 bp, synthetic construct
  source 1..20: mol_type = other DNA
ctccccagctaatcacacca

SEQ ID NO: 33 - DNA, 20 bp, synthetic construct
  source 1..20: mol_type = other DNA
tccaactaccacttgccagc

SEQ ID NO: 34 - DNA, 20 bp, synthetic construct
  source 1..20: mol_type = other DNA
gatgtgaaagtctcgggcgt

SEQ ID NO: 35 - DNA, 22 bp, synthetic construct
  source 1..22: mol_type = other DNA
tcaccatcttccaggagcgaga

SEQ ID NO: 36 - DNA, 21 bp, synthetic construct
  source 1..21: mol_type = other DNA
gaaggccatgccagtgagctt

SEQ ID NO: 37 - DNA, 3866 bp, synthetic construct
  source 1..3866: mol_type = other DNA
aaaccccaatcttcacctctgtggtcacaccaatttttgtttggtttctacagtgtctagctagctatgtttgggttcaaatagcctatgtatttattgcaatgttgggaactgaatgtagtttttgtttgtttgtttgttttttgcctaccaggcaagtacttgccattgagttataaccccaggcctttgtttacttttattatagacattttttttatgtgtgtgtgtgtgtgtgtgagagattgtgagtgcctttggaagctggaggaggacatcacctcccctggaactggagttacagtcgatggtgctggagcctgaactccagtcctctggaagcgcggcaagcactgaccactgagcattcagccctcttttgttttcttttggggatgggcccaggttggcctccaactcaagaggtagcctaggctgatgttcctaactccacctcctgaggcaaaagaccctgggggggcaaatgcctttaacttcagcacttgggaggcggaggcatgaggatctctgtgagttcgaggccagcctgatctacaaagtaagttccaagacagccagagctacacagagacactgtctccaaaagaaaaaaaaaaagaccctaattctaattcaggtcacatccacaatagaatagaacttgaacacatccttctggggacacacaattctacccactgcaggcaaacacaaaagagaaacaaggcagcccgttagcattctagtggtgacatgatgtgaagccaagtgggggtggcatgggagggtctggggcattgcagcctgggggagagcaccccagccagaggtgcagctggagcagaggcctgaggaaggaatgtacatgctggtttgaggagcttctaagaggctggggcatggggggctgagtggcagtaggagaggaagcgagccggagtgaaggagatggagcccatctaactcaggcctttgtcagctggtgagttcaagtacccacttcctgtctcaggtggcctctcagtcacaggctctggtgatttccctccttcccaccagacatctatgctattggggtgggcaagctggatgtggactggaaagaactgaatgagctgggttccaagaaggatggcgagaggcatgccttcatcttgcaggatgcaaaggccttgcaacagatctttgagcacatgttgggtgagtaagctttgtcccccgctgcagaagagagcatagtggggactcagatggggtctcacagtggcagcctggaccagtggcccttacccacttccctccccatcttcctttgcccatagatgtctctaagctcacagataccatctgtggggtggggaacatgtccgccaatgcctctgaccaggagaggacaccttggcaagtcacctttaaggtatcaggaaggagggacagggcttaggcatcagaggtaaaaacagccaggcacagcaaacccggattgttgtctcttccctgcagcccaagagcaaggaaacttgccagggatcactcatctctgatcagtgggtgctgacagcagctcactgcttccatgacattcagatggaggaccaccacctgtggagggtcaatgtaggtaagtcaggggctgcagtagatccctcactgcaaggccagagtcaccactgtctctcctcagcctttggtccagtctaattcacctttgtttccaggtgatcccacctctcagcatggcaaagaatttcttgtggaggacgtgataattgccccagggtttaatgtccatgcaaagcggaagcagggcatctcagagttctatgctgatgacattgccttgctgaagctatctcggaaagtgaaaatgtccacccatgccaggtgcctgaacccagatgggagagtaccctatagaggatggtgctctggaaagcaccagaggggatactgaggatgggcctgtttgacacttggctttctccccagacccatctgccttccttgcactgtgggagccaacatggctctgcggagatccccaggtagtacctgtaaagatcatggtgagtgctggaggcttgaggttcttggtgggttgcagccagagcttgcagggatcaggttcttgcagagtgccagcagggaccgggctgcagtcctcaagctgagtaaagaaatctgtaccaacacccacttctccccaatggcagagacagaacttctgtcacagcagaaagttcctgcacattttgtagctttgaatgggaacagactcaacatcaacctcaggacaggacctgaggtgagagcttagtaagggatgctgggataccctggaggcagctcccagaatgtccagccctgcctggagtctcgattcttggaccttacaggtctgcctaatgtctcctggaatgtcctcattcttctctcctatgccccacaccgcagtggacaaggtgtatccaggctgtctcccaaaacaaaaacatcttccccagcttgacaaacgttagcgaggtggtgacagaccagttcctatgcagtgggatggaggaggaagatgacaatccttgcaaaggttagtctgatcctggacttccagggagaaggctacggtgtccctgtaaccggttagcaagcactccaaatgctagtgtactgttctggacaatactgtcttttctttccctgaaggagaatctgggggagccgttttccttggacggagatacaggttcttccaggtgagaagcaggacccggaggggcctccctgccagggcacaagttcttcttgctgggggcaagtgggaggcctttgagaggaaccagagaggtcgaggcttagagtggggccaccactatctccaccctgttgtctcttccctccaggtgggcctggtgagttggggtctttttgacccttgtcatggttcctccaacaaaaacttgcgcaagaaacctccacgtggtgttctgccaagggacttccacattagtcttttccgcctgcagccctggctgaggcagcacctggatggtgtcctggactttctgccactttaacatggtcactgactcctttattagtctgaacttcctgtctaatacctctgagcgttctcactcctggatacataaatcttgggccccgggagcccagagacagtggcaaaagctagggaatccccaggattgtgccgggacctctgtgccacctgtgaagcaagtctctctctagtgtggatgacccgtgctccttttgctttcacacggaatttcccagttatgtaattaataaaaatcaatgatttccacatcctgtctgtcttatgtcttggggggtggggaggccaggaagattccaggaaggtcagagtccttgctgcacaaacagtggatggactttgctccatcacacagtccatggaaagactgatcttttaaattgggggtagtggaggtggtggtctgtgcttgttaggaggggtctgggggctaagagggagctttgaaagggaagttctggcccttggtcagtcaagggtggggctcacatagtttctgtttcctcagttggcagttcagctggggccctccttcatgaatgttccgggaagcagtggctgcgtgcgcagggtaggctggccaggctgcagatgccagagcagattgcataaaaggttaggggacagtgggaaaggggtgtagccagatccagcatttgggtttcagtttggacaggaggtcaaataggcacccagagtgacctggagagggctttgggccactggactctctggtgctttccatgacaatggagagcccccagctctgcctcgtcctcttggtcttaggctt

SEQ ID NO: 38 - DNA, 4077 bp, synthetic construct
  source 1..4077: mol_type = other DNA
cagaagacagggggagctaggctcccagtgcacttctttaggccagcttggaagctttctgggattattagtgtgtcaagtgacccatggcatacccttatctacacaggttggtgtgattagctggggagtagtagatgtctgcagagaccagaggcggcaacagctggtaccctcttatgcccgggacttccacatcaacctcttccaggtgctgccctggctaaaggacaagctcaaagatgaggatttgggttttctataaagagcttcctgcagggagagtgtgaggacagattaaagcagttacaataacaagtgtgttccacatctttttggggtaagggcgtgcactggttaacatcaacactgacagccgcttttgaaggcttaactccaatcccaagtgctgaaagactagaggctgacggaggtgaaaagcttctaccccaggattttactgagaccagcttgggggcatatgaggcacaaggaatccagcttcatgtcctagaagccatccacaaggtttcctatagatcgtcactgtacacaatctgggtcctcttgtctcgatggcaacccttagggctgttctggacagctaaggagggaggaaagtgacagttaagtgaagcaccagtggcgttagacctggggtccagagccctggccctggtccaccagggcttactctgccctctggtggccataacctcactgtggcttagaaaatccagaatgttaacacagttagagatgtgactatgataacatcacaaatacatggaaattaaaagatcagaatgtttctgtaccttgctggtacactggtcaattctggttccttcctagtgtgtgcaaggactttgcttactccttcctcagaaaagtttgttttgggtagaatgggctgtccacactgagagaccccatgaggacctctccgaactcaagtgttcagcttttctttcctcatactgctcatccctcccaaggattccctgtggggctaagagacaggcctcctctttggtcttatactcttttcagagcctctcagcccacagcccagagcttctggggttgttcttagcttggactcttcttcatggctcctttgctgcagacttaacttgggcctagcaagccaggactgctggaggtatgctaggcacagacagtagagcctagcttcctaatgctcttgattctctaaaccagtctcaggtcacttttcaatctccaaaatccccacctctgatggttccagatacacagaacactaatctatgtttccatgcctggtcttctacttgaggtccagacccacaataccaagttcaggtaacactccagctcagaggcgacaactaggcttctgctttcctgtctgtgacagaggaccctgttctgtttttccaaatggcttttcttttctttctttttttttttttggttttctgagacagggtttctctgtgtagtcttggctgtcctggaactcactctgtagaccaagctggccttgaactcagaaatccaccttcctctgcctcccaagtgctgggattaaaggtgtgtgccaccactgccctgcccaaatggcttttcaagacaagatttctctgtgtagccctggctgttctgaactctgctctgtagaccaggctggccttgaactcacctggctccacctcccacgtgttgtggctgaaggtgtgtgccaccactgagagggcacatttcagtgctgctctccttccctcacctgacagatgccctggcaattcttcatccactacctacgtgaagatcctgaccttgggcactttagggaactcaaggaagtgctatgctgcagagaggggaagggaggagcctcatccttaccaagggagccccagacagatttgccagtagcagcgtccagcatgggctgttttcgggctatgttgactttaagctgcacagattccacctgggtcccattgagctgtgggacaagaggggaggggacagaggacgggcattacatggagccaggtgctgctgccctgggagaccaaccaggaatgtgaggatgaaggttttctcagtcaggagaaaagtttcctctagaagcagatattgaaaagaagaagcaggaggatgacaggagggatgggaggaacggtctgagaagtcccaacctcagcaacagcctgatctgcagactccatcttctcgtaggtgacgaaggcacagctgggtgagagagaaagcagagtcaggaaactccatggagaccaggcagctccctccccgggatgttgctcatgcttactttctgggtgggtccatggagaggtcgatgatatttccaaagggagagaaggccccgcggaggagggtgggcgtcatgtcctctccatacacatacagtgtgttcccctttcgaggggccctccgttcggggaatgagtctgaccctgtgggttaggaaccacagtcattactgggtccacctcaccttctacttagcaggacccacctaaaccctggctaagatcactcactgcggaaagggccctctcggtctcgttcccgatctcggtcccggtctctgtctcgatcccggtctctgtctttgtctttatcccggtctctgtctcgatctcgatctcggtctctgtctctctctttgtcccgatccctatctcggctccggtcatgacttcggtccctgctgcggcttcggggaggggaggctgaggagcgggcgctaccatgctcttcatagctccagtcaaagcctcgaggtgggccatcaccagccccgggggcctctgcttcttctccatcttgtcccagttcccgaagccgatcactagaagacacaaagctggggagaggcagacagtaaggaccaaagggggttcgaccttcttccaaaccttgtggagtcaacactgcctctgcagctggctcctcccactctagccctgaactttccagtcactctggcctctgaccccacaccaaacggtgctctctctgacctttcatacagagatttcctctggggacgtctggatggctaaggggaaagaaaagacagagaacaattcaaatgattcccaggtgccggagttggtccacagtgtgtgggtctcttcttgtccccaaccctggccccacagaaaccattacctcctgtaggtcctcatcagcagacatgctcctctggaacggctggaaagtggggacaggccccttctctgggtcctggaaaagggcagatacccatgttagcgtggatcaggagagctcttccctctctcttctctgcttctcttttgctcctgtcactcttatgatgatgtgctggaccggttgactggtttttcaagatagtgcttctctgtgtggccctggctatcctgaacttgcgcagtagaaccaggctgtcctttatgttagagctctcggcctgtctgctccaagtgctgggattaaaggtgtgtgccactacatcagctgatgtgagtaactggtttcattactcaaacctcccttcaatccaagaagcacaaatatggaaaagagatgtgggcatcacccaggctttttttttttgttttgtttttttttgttttgtttttcgagacagggtttctctgtatagccctggctgtcctagaactcactctgtagaccgggctggcctcaaactcagaaatctgcctgcctctgccccacaagtgctgggattaaaggcatgtgccaccacactgggctcaggtttctttgtgatagacagaaacctagcgctccagtgggctgcagtggcaaaaactacttctgaggctgaggccagagcatcacttgactccatgagtacagtcagaccctgtctcaaggaacaagaaagaaacaccctaaactcagaacagcacaggttgctcatatgtgagcatgcatgacttcccccacccacccccttccagctgatgccaggacgttccagacaatcttcctgtgtgctcacctttaacttcccttccagggtccgagaacgtttgaagcctgagttct

SEQ ID NO: 39 - DNA, 12990 bp, synthetic construct
  source 1..12990: mol_type = other DNA
aattattatttttaatcaacagctttagacagagaaccttggtttcatcttcagtgggctgtggccatgggcagtttcttcatctgcaaaaggggagtagtactaggacccagctcacaagctgacaggggaagatgctcagacaaacactgcctgcctggcatagaaaaatgcccagcatatgttagccatgaccacgaccgtcgtcgttatcatcatcatcatcatcatagcatctcatgtttcaggaaactttccaggaagaagggacctcgattccctctggggaatgtccctggtggttgctctttcagcagcacagctggctaactaaggctttggcagttgcagcctctaaaggaaaaattcctcaggttcagactaaacacaaattgcactgacctttgatcagaaagtaatttcagagagagagatgctcagacagggagggcagctggttttgagccccaacctttcatcttccccttagctcctctcctttccattcacactgccccctcccccatcacctggccctcgggggtaagctgattcctctttaaaactctggcccaaggaagacaaaatttaaagcccactcccttcctccttagcatcactggaccaaggtcaaatgctacaaaaacattttattgaaaataagcaggaaaccaaacgaaaatagtcaaagaaaacgcacaaggcacgatcgttgtctagctccaactgtaactgtttctatctgggccattgccagattgcctcctggctgaagatctcttggtccacctaagcaccttgctttttacacacaacgcggggctctctgagaacaaaaatgggccacaaggggtgcaaaggctgggagaggagtagactctgtggtctgtctgagggcagttctgactggcaccacagtcggaggacaggcgcggcctgttgtgtgggtccagggcctccagtgggaaaacgtggctttaggcccttctcccagatgctaccttttacagaggaagaccagatctgaggtttagtttccatgttgtgttctgagttctttctattcattcagtcatttaaaagtacttaccaaactaccacaaacctgggtggcttagaacacagaatttctttttcttacagttctggaggttagaagtctgaaatcaaggtgttggcagggccgtgcttcctcagaaggctcttgggaagaattctttcctgccttttccggctgccggcagctccaaccttggcttgcggcagcataaacccattctctgcctctgtcttcaactcgccttcttttctgtgtgtgcctctgtgtcattacatgctgttctcttatatagataggagacccactacctgtgtctttgtgtccaaattcctttcttctttttctgttcatttgtttgagacagagtctcgctctgtcacccagaagcccaggctgcagtgcagtggcgggatcccggctcactgtaacctctgcctcctgggttcaggtgattctcgtgcctcagtctcccaagaagctgggattacaggcatgtgccaccatgcccggcaaatttttgtatttttagtagagacatggtctcgccatgttggctaggctggtcttaaactcctggcctcaaggcgatctgcctgccttcgcctcaaaaaaactgccgggattacaggcatgagtcaccaccatgcccagccagttcacttttttttttttttttttttttgagatggagtcttgctctgttgcccaggctggagtgcagtggtgcaatctcggctcactgcaacatccgcctcccggttcaagcgattctcctgcctcagcctcctgagtagctgggattacaggtgtgtgccagcatgtctggctaatttttgtatttttagtagagacagggtttcaccatgttggtcaggctggtcttgaattcctgacctcgtgatctgcccgcctcagcctcccagagtgctgggattacaggtgtgagccaccgtgcccggctcacctcttctttttttttttttgagacggggttttgctcttgttgcccaggctggagtgcaatggcgcgatcttggctcaccacaaccaccgcctcctggtgattacaggtgtgagccaccacgcctggctctggcttacctcttcttataaggacctcagtcattggattagagctcaccctaatctagtatgacttaatcttaacttgattacatctgcaaagaccctttttccaaataaagtcacagatactggggattaggactcgaacacatctttctgggggacacaattccaccattacagggaataaacaggataagaaaaccatagaacccagcaggtggtaggtgacacaagctaaggggtgttgccatgttgcccaggctggtctcaaacttctggcttcaagggatcctcccaccttgcctcccaaagtggggatgaaagtttgtctggggcattgcagttttagacaggaagaccagggaaggcctcactgagaaggtgacatttgagccaagacttaaaaaggtacgaaagtgagccatgtggaagtctgggggggaggagtgaactaggcagaggcacagctgggcaaagggcctgaggtgtgaccatgcctatggatttgaggaacttcaaagaggctgtgtgctgcaggagagtgaagggcagggagtggcaggaaatgaaggcagacaggtagcagtggggaggacgcaggggtccagctcatgtaggtcttgattggacacagtgagtttcagatgacagcctcctgtctcatggggtagccccaaagccacaggagtctggtgatttccctcttccccaccagacatctatgccatcggggtgggcaagctggatgtggactggagagaactgaatgagctagggtccaagaaggatggtgagaggcatgccttcattctgcaggacacaaaggctctgcaccaggtctttgaacatatgctgggtgagtgagctttgccctccttggtgtggggaggatggtgaggagcccgccagaggcccgtgttgggaacctggacacagtgcccctcacttgcctccttccccatctgatcctcacacccacagatgtctccaagctcacagacaccatctgcggggtggggaacatgtcagcaaacgcctctgaccaggagaggacaccctggcatgtcactattaaggtaccaggaaggaggggcagggcttggattccagaggtaaaagcggccatgggccagacatactgcaatctctgaaaatcacctgttcccctgcagcccaagagccaagagacctgccggggggccctcatctccgaccaatgggtcctgacagcagctcattgcttccgcgatggcaacgaccactccctgtggagggtcaatgtgggtaaggcaggggatgcaccagcctcctgatcctgaagccacagatcctaccacctcacccagcctctggcccctgcaggagccctggtctagcctaatctagtgtatcatttccaggagaccccaaatcccagtggggcaaagaattccttattgagaaggcggtgatctccccagggtttgatgtctttgccaaaaagaaccagggaatcctggagttctatggtgatgacatagctctgctgaagctggcccagaaagtaaagatgtccacccatgccaggtgcctggagtctgggatgggagggtgccctgcagggaagagtgctctggagatccctggaagagatactggggacaggctggtgtgacccttgctcttctccccaggcccatctgccttccctgcacgatggaggccaatctggctctgcggagacctcaaggcagcacctgtagggaccatggtgagtgctgggacttatggtgcttgagagctggggccggggtttgggggtgataacaaggactaggctgcagtccccaagccaggaacctggattctgggtaaaaggaccagcaccaacatccccttctcttgactatagagaatgaactgctgaacaaacagagtgttcctgctcattttgtcgccttgaatgggagcaaactgaacattaaccttaagatgggagtggaggtgagggtctcaggttggggatgctgggatccccctgtgacagctcccagaatgtctctcttccttctccaggtctggctgctttctctctctgacgcgggtcacccctcctcccaagcctcacaaacctgctaggtgtccctgggtctgcttattctttttttgttgttattgagatggagtcttgctctgtctcccaggctggagtgcagtggcacgacctcagctcactgcaacttctgcctcctgggttcaagcgattctcctacttcagcctcccgagtagctgagattacaggtgcccaccaccacaccagctaatttttgtatttttagtagagacgggatttcgccatgttggccaggatggtcttgaactcctgacctcaagtgatctgcctgcctcaacctcccaaagtgctgagattacaggcgtgagccactgcacccacccgggtctgcttattctacccttctctctggttccacccctgctgcagtggacaagctgtgccgaggttgtctcccaagaaaaaaccatgttccccaacttgacagatgtcagggaggtggtgacagaccagttcctatgcagtgggacccaggaggatgagagtccctgcaagggtgagtccctcaccatgcctggattcccaaggggaaggccacctgtgtctctgtggccagcatgcatgccagaacaccagtccactgccctagatgacactgtctcctgtcaccctttgctggcaggagaatctgggggagcagttttccttgagcggagattcaggttttttcaggtgagaaggtagaagcttgcaggacccaggggttacaggatctcagccttgttggggggatgagggaggcctttgagggatctagggaggttggggcttacagttggggctgtggcagcctcccagccagttctctccttttctccaggtgggtctggtgagctggggtctttacaacccctgccttggctctgctgacaaaaactcccgcaaaagggcccctcgtagcaaggtcccgccgccacgagactttcacatcaatctcttccgcatgcagccctggctgaggcagcacctgggggatgtcctgaattttttacccctctagccatggccactgagccctctgctgccctgccagaatctgccgcccctccatcttctacctctgaatggccacccttagaccctgtgatccatcctctctcctagctgagtaaatccgggtctctaggatgccagaggcagcgcacacaagctgggaaatcctcagggctcctaccagcaggactgcctcgctgccccacctcccgctccttggcctgtccccagattccttccctggttgacttgactcatgcttgtttcactttcacatggaatttcccagttatgaaattaataaaaatcaatggtttccacatctctcagtgcctctatctggaggccaggtagggctggccttgggggagggggaggccagaatgactccaagagctacaggaaggcaggtcagagaccccactggacaaacagtggctggactctgcaccataacacacaatcaacaggggagtgagctggatccttatttctggtccctaagtgggtggtttgggcttactggggaggagctaaggccggagaggaggtactgaaggggagagtcctggacctttggcagcaaagggtgggacttctgcagtttctgtttccttgactggcagctcagcggggccctcccgcttggatgttccgggaaagtgatgtgggtaggacaggcggggcgagccgcaggtgccagaacacagattgtataaaaggctgggggctggtggggagcaggggaagggaatgtgaccaggtctaggtctggagtttcagcttggacactgagccaagcagacaagcaaagcaagccaggacacaccatcctgccccaggcccagcttctctcctgccttccaacgccatggggagcaatctcagcccccaactctgcctgatgccctttatcttgggcctcttgtctggaggtaagcgagggtaaccttcccttcctgctgtctccagcatccctccttggccttttggggccaggcttcatcagcctttctcttcaggtgtgaccaccactccatggtctttggcccggccccagggatcctgctctctggagggggtagagatcaaaggcggctccttccgacttctccaagagggccaggcactggagtacgtgtgtccttctggcttctacccgtaccctgtgcagacacgtacctgcagatctacggggtcctggagcaccctgaagactcaagaccaaaagactgtcaggaaggcagagtgcagaggtttgagggcaatgagtgtgggcagtggcctaaggcagaaacagggcaggcggcagcaaggtcaggactaggatgagactaggcagggtgacaaggtgggctgaccgggagtaggagcagttttagggtggcaggcggaaagggggcaagaaaaagcggagttaacccttactaagcatttaccctgggcttccaggcagccctggaagtcaagagaacactcagaaatggggagggagaagcagtggaaatccatatgggttgaggagtaggtaagatgctgcttctgcgggactgggaatgcgctgtttctcagtgacatggtctccgagaccaggagggatacacctaaggcagcctttccctcttgatgacttctacttgtccccccttctcaaagcaatccactgtccaagaccacacgacttcgagaacggggaatactggccccggtctccctactacaatgtgagtgatgagatctctttccactgctatgacggttacactctccggggctctgccaatcgcacctgccaagtgaatggccgatggagtgggcagacagcgatctgtgacaacggaggtgagaagcatcccctccccctacattgctgtctccctgacggcgcccagcccgaggagtgggcactcggctccggacactgtaactcttgctctctaccttgctcacggggcctcaggcttcagtgcttacctcgatgtctcatacctctgcagcggggtactgctccaacccgggcatccccattggcacaaggaaggtgggcagccagtaccgccttgaagacagcgtcacctaccactgcagccgggggcttaccctgcgtggctcccagcggcgaacgtgtcaggaaggtggctcttggagcgggacggagccttcctgccaaggtgacctttgacctgtacccccaggtcagatcctggtcttccatcctactgtcttctctccccacctcaaccctgctctttcctcactttgtttaaacctccctgtacaactatctcacttctgagccttttataccctggaaacccatgatcccccgtctctttggtcactgtatccctgacactcccagacatttgacctcatttctgactctcccagactccttcatgtacgacacccctcaagaggtggccgaagctttcctgtcttccctgacagagaccatagaaggagtcgatgctgaggatgggcacggcccaggtttgaagacagagaagggaggcagggcagggaactgggggaaaatggagaagggacagaactgttaatgctggagcctgagccactctcctggcacccaggggaacaacagaagcggaagatcgtcctggacccttcaggctccatgaacatctacctggtgctagatggatcagacagcattggggccagcaacttcacaggagccaaaaagtgtctagtcaacttaattgagaaggtggaatcctcctatccctgaactcgggggaatggaatctcgctgatcttccaggactagctccctgatcattccagcccctctgaacaacagggccccaggaaaatctccaggtcctattctgtcctccttcccttttacttgaagcagtttcttgactggtaattcctccatgaacctcagcccttgagcctcttactgagagcctccctgtcccagcaaagtcgctgaaatctcccaatcacagtattctattttcaatgccatggcgccttgttctcctcacccacaggtggcaagttatggtgtgaagccaagatatggtctagtgacatatgccacataccccaaaatttgggtcaaagtgtctgaagcagacagcagtaatgcagactgggtcacgaagcagctcaatgaaatcaattatgaaggtcagaggttagggaatggtgggaggttcactttggggtcaggaggttcagggtggagggggtcatgagactaccttgagggcgacagggaggaccactttgtagtcaaaagttgaacagcaggatcgttgggcaatggaggttagtgggaacctgttgggggctggaagggccactttgtggtcaaagggaagtccgtgtaatgatgattaacttaaaaagttgaaagatgtgggatttcagttgcagattggtctctggggttaaaagatggcttggaagaccaggtgaggtgatggtctcttccctctccacagaccacaagttgaagtcagggactaacaccaagaaggccctccaggcagtgtacagcatgatgagctggccagatgacgtccctcctgaaggctggaaccgcacccgccatgtcatcatcctcatgactgatggtcagaagggacctctctcctgtcccagcctccccaccttctcagaccagcatgtggcccttaagtccacttgtaacactatacccatggttggggccctgaatgtgactcatagctggctgttcatctctcctgtgacccttcataaggaattcttcctaagccctgtgatcaactatctctaacccttcctcaacttgctcaccctgccatgtgtatccctgcctttagccagtttatcttccttatctcctaccctcatggtcctgtctcttctgcaggattgcacaacatgggcggggacccaattactgtcattgatgagatccgggacttgctatacattggcaaggatcgcaaaaacccaagggaggattatctgggtgagtaacctgcctaggacccagcaccccacttcctcagggcttggaccctcatccttcctttttatccctcagatgtctatgtgtttggggtcgggcctttggtgaaccaagtgaacatcaatgctttggcttccaagaaagacaatgagcaacatgtgttcaaagtcaaggatatggaaaacctggaagatgttttctaccaaatgatcggtagggagatacaagggaataaagaacacaactctcctcaggttcccctgaagtaattcattcttcctctacacctgaagctctagttgcctggaaagccttcttcattcctccttctctacctcagtgtcactattcttgtttcctggcactgttcacttaaccttagaatcacagagctctgagcacttcagagatctttctatagtcctacatttgacacgtggaaacagaagccaaaggaggtcaagggacagcaagttagcaacaagggtgggcttgaaaacagccaggcctctgacagcttgatcccaagttctttcccttttcagtccaccatagcagttttctcctaacacgaggaaacaaatacccgtggtctttccctttctccttttgggcctttgctccccatagactcctacccaaaaggctgctgccatttgggaatgaagtgttccgagttttcagcacattctccttctctgccagatgaaagccagtctctgagtctctgtggcatggtttgggaacacaggaagggtaccgattaccacaagcaaccatggcaggccaagatctcagtcattgtaagcacagaatcccagtagtggggacttgggggaggtgaggtcaaggtgaaatgggagtaggggaaggaaaaaatggccataagagatggtggtttgtgaaagttgagctttccctctctactgttgtgtccccagcgcccttcaaagggacacgagagctgtatgggggctgtggtgtctgagtactttgtgctgacagcagcacattgtttcactgtggatgacaaggaacactcaatcaaggtcagcgtaggtaaggatgcaactgaaggtcctgggctgcacctatgctctccaggcaacacctcccactttctacagatcctacactccacccatcctcaatgcagccccattccttgcaccccagaccagtcagggatgggggaagacgtgaagttaggaatgacacggggccagaggcaggaagctgcccacaaagaggtggtacctactctcctacttcaggaggggagaagcgggacctggagatagaagtagtcctatttcaccccaactacaacattaatgggaaaaaagaagcaggaattcctgaattttatgactatgacgttgccctgatcaagctcaagaataagctgaaatatggccagactatcaggtgagagcgtccagatccctgaggaaaggctgggaaaggctggaggactggggtgaggagcaggcctggtttgctgttctccttgtcctttataggcccatttgtctcccctgcaccgagggaacaactcgagctttgaggcttcctccaactaccacttgccagcaacaaagtaagacatacttggcaagaggataaggatgagatcccaagagacaagtggggcatgagagggaggtgcaataggaagagatgatgcctggcccagaacctagctctagaagggcttaggggacatctactgagtgacaaaggcaatggggagatgacagtggtgggagcagctgaagtgacgcagtctattcgtccagaggaagagctgctccctgcacaggatatcaaagctctgtttgtgtctgaggaggagaaaaagctgactcggaaggaggtctacatcaagaatggggataaggtgagaaacgggcatcctaaggaggcactctaggccccaatccttcctaagccacttctgttcattacttctccatgcttcccacctcccctacagaaaggcagctgtgagagagatgctcaatatgccccaggctatgacaaagtcaaggacatctcagaggtggtcacccctcggttcctttgtactggaggagtgagtccctatgctgaccccaatacttgcagaggtgagagaatgctctttggttgtgctacaagtgcccaaggcccaacagtccttttctctacagcttctcctctccttgcaggtgattctggcggccccttgatagttcacaagagaagtcgtttcattcaagtgagtcctccctttcctatctggggagatgccaagtggtcagcatgggccccaaagcaggaaagctcaatgcatgtggctagtaattcgaggtaggcagagcctgcctcaccttaggaccgcatgtcttgcctgcgtgtgtcaagaacgaggctgagctgggtccctagtctgattcctttaggtcagctaagacacaagcaggaacagccatgcttccaggattaggaattctactgaatgatccatggcaccccactgcctctgcaggttggtgtaatcagctggggagtagtggatgtctgcaaaaaccagaagcggcaaaagcaggtacctgctcacgcccgagactttcacatcaacctctttcaagtgctgccctggctgaaggagaaactccaagatgaggatttgggttttctataaggggtttcctgctggacaggggcgtgggattgaattaaaacagctgcgacaacacctgtgttccagatccttttggggcaagggagtggggaacaggcactggccatgttgttacactgagatcaaacctgacagccgtttttaaaggtttaaccccaatcccaagtgctgaaaaaccagaggctgagggagatgtgtaagcttccacctcagtgttttactgagaccagcattggggcatatgaggcacaaggaatccagctctgttccctagaagccatccacaaggttttccttgtagacgtcatcactgtagacaatctgggtcctcttgtcccggtggcaacccttagggctgttctggacagctagggagggaggagaggaacagttaaggtctaaaggagatcatagaacagaccctgaggctgactcctgaccacctcactcctggccactggcccctggaagcccagtttccacgctgccctctggtggccaggatggcctgtcttccttagctcctttgtgccaacccatggccaagaaaagtataagtggacattttgatgaatgttttgttcttagaaaaatcccaaatgtcattgttgagacacgtgaatgatattaacccactacttacagtcagtatgtcagaagctaaaaactagaaaacctctgtagcccttttttgacatgctggtcaattctagttcctttcttttgcctgaagggccactgtagctgagcccttctttctgctcactcctttcccaggaaaatctactttcagggaaaatggattattcacactaagaaatgctactagctccaccagaactcattcagggtgtagctttggccctcaccattctctctcaagcctctagctgtttcttccccttcctctttcctccctccaccagacatgttactctcttcaccccatccaatggttccatccccaccacccttgagctacagagaatctctctcacccactcccatcctgtgatctctgtgcctcaacactgctggctactccctctttctc

SEQ ID NO: 40 - RNA, 2476 nt, synthetic construct
  source 1..2476: mol_type = other RNA
gggaagggaatgtgaccaggtctaggtctggagtttcagcttggacactgagccaagcagacaagcaaagcaagccaggacacaccatcctgccccaggcccagcttctctcctgccttccaacgccatggggagcaatctcagcccccaactctgcctgatgccctttatcttgggcctcttgtctggaggtgtgaccaccactccatggtctttggcccggccccagggatcctgctctctggagggggtagagatcaaaggcggctccttccgacttctccaagagggccaggcactggagtacgtgtgtccttctggcttctacccgtaccctgtgcagacacgtacctgcagatctacggggtcctggagcaccctgaagactcaagaccaaaagactgtcaggaaggcagagtgcagagcaatccactgtccaagaccacacgacttcgagaacggggaatactggccccggtctccctactacaatgtgagtgatgagatctctttccactgctatgacggttacactctccggggctctgccaatcgcacctgccaagtgaatggccgatggagtgggcagacagcgatctgtgacaacggagcggggtactgctccaacccgggcatccccattggcacaaggaaggtgggcagccagtaccgccttgaagacagcgtcacctaccactgcagccgggggcttaccctgcgtggctcccagcggcgaacgtgtcaggaaggtggctcttggagcgggacggagccttcctgccaagactccttcatgtacgacacccctcaagaggtggccgaagctttcctgtcttccctgacagagaccatagaaggagtcgatgctgaggatgggcacggcccaggggaacaacagaagcggaagatcgtcctggacccttcaggctccatgaacatctacctggtgctagatggatcagacagcattggggccagcaacttcacaggagccaaaaagtgtctagtcaacttaattgagaaggtggcaagttatggtgtgaagccaagatatggtctagtgacatatgccacataccccaaaatttgggtcaaagtgtctgaagcagacagcagtaatgcagactgggtcacgaagcagctcaatgaaatcaattatgaagaccacaagttgaagtcagggactaacaccaagaaggccctccaggcagtgtacagcatgatgagctggccagatgacgtccctcctgaaggctggaaccgcacccgccatgtcatcatcctcatgactgatggattgcacaacatgggcggggacccaattactgtcattgatgagatccgggacttgctatacattggcaaggatcgcaaaaacccaagggaggattatctggatgtctatgtgtttggggtcgggcctttggtgaaccaagtgaacatcaatgctttggcttccaagaaagacaatgagcaacatgtgttcaaagtcaaggatatggaaaacctggaagatgttttctaccaaatgatcgatgaaagccagtctctgagtctctgtggcatggtttgggaacacaggaagggtaccgattaccacaagcaaccatggcaggccaagatctcagtcattcgcccttcaaagggacacgagagctgtatgggggctgtggtgtctgagtactttgtgctgacagcagcacattgtttcactgtggatgacaaggaacactcaatcaaggtcagcgtaggaggggagaagcgggacctggagatagaagtagtcctatttcaccccaactacaacattaatgggaaaaaagaagcaggaattcctgaattttatgactatgacgttgccctgatcaagctcaagaataagctgaaatatggccagactatcaggcccatttgtctcccctgcaccgagggaacaactcgagctttgaggcttcctccaactaccacttgccagcaacaaaaggaagagctgctccctgcacaggatatcaaagctctgtttgtgtctgaggaggagaaaaagctgactcggaaggaggtctacatcaagaatggggataagaaaggcagctgtgagagagatgctcaatatgccccaggctatgacaaagtcaaggacatctcagaggtggtcacccctcggttcctttgtactggaggagtgagtccctatgctgaccccaatacttgcagaggtgattctggcggccccttgatagttcacaagagaagtcgtttcattcaagttggtgtaatcagctggggagtagtggatgtctgcaaaaaccagaagcggcaaaagcaggtacctgctcacgcccgagactttcacatcaacctctttcaagtgctgccctggctgaaggagaaactccaagatgaggatttgggttttctataaggggtttcctgctggacaggggcgtgggattgaattaaaacagctgcgacaaca

SEQ ID NO: 41 - DNA, 94 bp, synthetic construct
  source 1..94: mol_type = other DNA
tgacaatggagagcccccagctctgcctcgtcctcttggtcttaggcttaattattatttttaatcaacagctttagacagagaaccttggttt

SEQ ID NO: 42 - DNA, 86 bp, synthetic construct
  source 1..86: mol_type = other DNA
gatctctgtgcctcaacactgctggctactccctctttctcgaagttcctattctctagaaagtataggaacttcaggtctgaaga

SEQ ID NO: 43 - DNA, 85 bp, synthetic construct
  source 1..85: mol_type = other DNA
ccatcctgtgatctctgtgcctcaacactgctggctactccctctttctcgaagttcctattctctagaaagtataggaacttca

SEQ ID NO: 44 - DNA, 75 bp, synthetic construct
  source 1..75: mol_type = other DNA
gaagttcctattctctagaaagtataggaacttccagaagacagggggagctaggctcccagtgcacttctttag

SEQ ID NO: 45 - DNA, 1264 bp, synthetic construct
  source 1..1264: mol_type = other DNA
ttccagggagaaggctacggtgtccctgtaaccggttagcaagcactccaaatgctagtgtactgttctggacaatactgtcttttctttccctgaaggagaatctgggggagccgttttccttggacggagatacaggttcttccaggtgagaagcaggacccggaggggcctccctgccagggcacaagttcttcttgctgggggcaagtgggaggcctttgagaggaaccagagaggtcgaggcttagagtggggccaccactatctccaccctgttgtctcttccctccaggtgggcctggtgagttggggtctttttgacccttgtcatggttcctccaacaaaaacttgcgcaagaaacctccacgtggtgttctgccaagggacttccacattagtcttttccgcctgcagccctggctgaggcagcacctggatggtgtcctggactttctgccactttaacatggtcactgactcctttattagtctgaacttcctgtctaatacctctgagcgttctcactcctggatacataaatcttgggccccgggagcccagagacagtggcaaaagctagggaatccccaggattgtgccgggacctctgtgccacctgtgaagcaagtctctctctagtgtggatgacccgtgctccttttgctttcacacggaatttcccagttatgtaattaataaaaatcaatgatttccacatcctgtctgtcttatgtcttggggggtggggaggccaggaagattccaggaaggtcagagtccttgctgcacaaacagtggatggactttgctccatcacacagtccatggaaagactgatcttttaaattgggggtagtggaggtggtggtctgtgcttgttaggaggggtctgggggctaagagggagctttgaaagggaagttctggcccttggtcagtcaagggtggggctcacatagtttctgtttcctcagttggcagttcagctggggccctccttcatgaatgttccgggaagcagtggctgcgtgcgcagggtaggctggccaggctgcagatgccagagcagattgcataaaaggttaggggacagtgggaaaggggtgtagccagatccagcatttgggtttcagtttggacaggaggtcaaataggcacccagagtgacctggagagggctttgggccactggactctctggtgctttccatgacaatggagagcccccagctctgcctcgtcctcttggtcttaggctt

SEQ ID NO: 46 - DNA, 1318 bp, synthetic construct
  source 1..1318: mol_type = other DNA
cagaagacagggggagctaggctcccagtgcacttctttaggccagcttggaagctttctgggattattagtgtgtcaagtgacccatggcatacccttatctacacaggttggtgtgattagctggggagtagtagatgtctgcagagaccagaggcggcaacagctggtaccctcttatgcccgggacttccacatcaacctcttccaggtgctgccctggctaaaggacaagctcaaagatgaggatttgggttttctataaagagcttcctgcagggagagtgtgaggacagattaaagcagttacaataacaagtgtgttccacatctttttggggtaagggcgtgcactggttaacatcaacactgacagccgcttttgaaggcttaactccaatcccaagtgctgaaagactagaggctgacggaggtgaaaagcttctaccccaggattttactgagaccagcttgggggcatatgaggcacaaggaatccagcttcatgtcctagaagccatccacaaggtttcctatagatcgtcactgtacacaatctgggtcctcttgtctcgatggcaacccttagggctgttctggacagctaaggagggaggaaagtgacagttaagtgaagcaccagtggcgttagacctggggtccagagccctggccctggtccaccagggcttactctgccctctggtggccataacctcactgtggcttagaaaatccagaatgttaacacagttagagatgtgactatgataacatcacaaatacatggaaattaaaagatcagaatgtttctgtaccttgctggtacactggtcaattctggttccttcctagtgtgtgcaaggactttgcttactccttcctcagaaaagtttgttttgggtagaatgggctgtccacactgagagaccccatgaggacctctccgaactcaagtgttcagcttttctttcctcatactgctcatccctcccaaggattccctgtggggctaagagacaggcctcctctttggtcttatactcttttcagagcctctcagcccacagcccagagcttctggggttgttcttagcttggactcttcttcatggctcctttgctgcagacttaacttgggcctagcaagccaggactgctggaggtatgctaggcacagacagtagagcctagcttcctaatgctcttgattctctaaaccagtctcaggtcacttttcaatctccaaaatccccacctctgatggttccagatacacagaacactaatctatgtttccatgcctggtcttctactt

SEQ ID NO: 47 - DNA, 23 bp, synthetic construct
  source 1..23: mol_type = other DNA
tgcaggttcgagtctgcacgggg

SEQ ID NO: 48 - DNA, 23 bp, synthetic construct
  source 1..23: mol_type = other DNA
tcttctacaggagattccggggg

SEQ ID NO: 49 - RNA, 20 nt, synthetic construct
  source 1..20: mol_type = other RNA
tgcaggttcgagtctgcacg

SEQ ID NO: 50 - RNA, 24 nt, synthetic construct
  source 1..24: mol_type = other RNA
taggtgcaggttcgagtctgcacg

SEQ ID NO: 51 - RNA, 20 nt, synthetic construct
  source 1..20: mol_type = other RNA
cgtgcagactcgaacctgca

SEQ ID NO: 52 - RNA, 24 nt, synthetic construct
  source 1..24: mol_type = other RNA
aaaccgtgcagactcgaacctgca

SEQ ID NO: 53 - RNA, 20 nt, synthetic construct
  source 1..20: mol_type = other RNA
tcttctacaggagattccgg

SEQ ID NO: 54 - RNA, 24 nt, synthetic construct
  source 1..24: mol_type = other RNA
taggtcttctacaggagattccgg

SEQ ID NO: 55 - RNA, 20 nt, synthetic construct
  source 1..20: mol_type = other RNA
ccggaatctcctgtagaaga

SEQ ID NO: 56 - RNA, 24 nt, synthetic construct
  source 1..24: mol_type = other RNA
aaacccggaatctcctgtagaaga

SEQ ID NO: 57 - protein, 763 aa, Rattus norvegicus
MTMEGPQLCLVLLVLGLSSGGVSATPVLEARPQVSCSLEGVEIKGGSFQLLQDGQALEYLCPSGFYPYPVQTRTCKSTGSWSVLQTRDQKIVKKAECRAIRCPRPQDFENGEFWPRSPYYNLSDQISFQCYDGYTLRGSANRTCQENGRWDGQTAICDDGAGYCPNPGIPIGTRKVGSQYRLEDTVTYHCSRGLVLRGSQQRRCQEGGSWSGTEPSCQDSFMYDSPQEVAEAFLSSLTETIEGADAEDGHSPGEQQKRKIILDPSGSMNIYMVLDGSDSIGASNFTGAKRCLANLIEKVASYGVKPRYGLVTYATVPKVLVRVSEERSSDADWVTEKLNQISYEDHKLKSGTNTKKALQAVYSMMSWPGDAPPEGWNRTRHVIIIMTDGLHNMGGDPVTVIEDIRDLLDIGRDRKNPREDYLDVYVFGVGPLVDPVNINALASKKNNEQHVFKVKDMEDLENVFYKMIDETKSLGLCGMVWEHQKGGDYYKQPWQAKISVTRPLKGHENCMGAVVSEYFVLTAAHCFTVEDQKHSIKVNVEGKRRDLEIEEVLFHPNYDINGKKAEGISEFYDYDVALIKLKTKLKYSQTLRPICLPCTEGTTRALRLPQTATCKQHKEELLPMKDVKALFVSEEGKKLTRKEVYIKNGEKKASCERDATKAQGYEKVKVASEVVTPRFLCTGGVDPYADPNTCKGDSGGPLIVHKRSRFIQVGVISWGVVDVCKDPRRQQLVPSYARDFHINLFQVLPWLKEKLKDEDLGFL

SEQ ID NO: 58 - RNA, 21 nt, synthetic construct
  source 1..21: mol_type = other RNA
  modified_base 1..8: mod_base = OTHER; note = 2'-O-methyl
  modified_base 1^2: mod_base = OTHER; note = phosphorothioate linkage
  modified_base 2^3: mod_base = OTHER; note = phosphorothioate linkage
  modified_base 9..11: mod_base = OTHER; note = 2'-fluoro modification
  modified_base 12..21: mod_base = OTHER; note = 2'-O-methyl
gaattcctgaattttatgact

SEQ ID NO: 59 - RNA, 23 nt, synthetic construct
  source 1..23: mol_type = other RNA
  modified_base 1: mod_base = OTHER; note = 2'-O-methyl
  modified_base 2: mod_base = OTHER; note = 2'-deoxyguanosine-3'-phosphate
  modified_base 3..4: mod_base = OTHER; note = 2'-O-methyl
  modified_base 5: mod_base = OTHER; note = 2'-deoxyadenosine-3'-phosphate
  modified_base 6: mod_base = OTHER; note = 2'-O-methyl
  modified_base 7: mod_base = OTHER; note = 2'-deoxyadenosine-3'-phosphate
  modified_base 8..11: mod_base = OTHER; note = 2'-O-methyl
  modified_base 12: mod_base = OTHER; note = 2'-deoxythymidine-3'-phosphate
  modified_base 12: mod_base = OTHER; note = Thymine
  modified_base 13: mod_base = OTHER; note = 2'-O-methyl
  modified_base 14: mod_base = OTHER; note = 2'-fluoro modification
  modified_base 15..23: mod_base = OTHER; note = 2'-O-methyl
  modified_base 1^2: mod_base = OTHER; note = phosphorothioate linkage
  modified_base 2^3: mod_base = OTHER; note = phosphorothioate linkage
  modified_base 21..22: mod_base = OTHER; note = phosphorothioate linkage
  modified_base 22..23: mod_base = OTHER; note = phosphorothioate linkage
agtcataaaattcaggaattcct